European Patent Application EP 4 589 008 A1, published July 23, 2025. Title: A double-stranded circular DNA vector, a method for producing linear covalently closed DNA, and a fusion polypeptide comprising a protelomerase and an endonuclease. Applicant: KANEKA CORPORATION. Application JP. The sequence listing filed with the application follows.

SEQUENCE LISTING (38 sequences)

SEQ ID NO: 1 - DNA, 2637 bp, synthetic construct
  source 1..2637: mol_type = other DNA
atgagcaaggtaaaaatcggtgagttgatcaacacgcttgtgaatgaggtagaggcaattgatgcctcagaccgcccacaaggcgacaaaacgaagagaattaaagccgcagccgcacggtataagaacgcgttatttaatgataaaagaaagttccgtgggaaaggattgcagaaaagaataaccgcgaatacttttaacgcctatatgagcagggcaagaaagcggtttgatgataaattacatcatagctttgataaaaatattaataaattatcggaaaagtatcctctttacagcgaagaattatcttcatggctttctatgcctacggctaatattcgccagcacatgtcatcgttacaatctaaattgaaagaaataatgccgcttgccgaagagttatcaaatgtaagaataggctctaaaggcagtgatgcaaaaatagcaagactaataaaaaaatatccagattggagttttgctcttagtgatttaaacagtgatgattggaaggagcgccgtgactatctttataagttattccaacaaggctctgcgttgttagaagaactacaccagctcaaggtcaaccatgaggttctgtaccatctgcagctaagccctgcggagcgtacatctatacagcaacgatgggccgatgttctgcgcgagaagaagcgtaatgttgtggttattgactacccaacatacatgcagtctatctatgatattttgaataatcctgcgactttatttagtttaaacactcgttctggaatggcacctttggcctttgctctggctgcggtatcagggcgaagaatgattgagataatgtttcagggtgaatttgccgtttcaggaaagtatacggttaatttctcagggcaagctaaaaaacgctctgaagataaaagcgtaaccagaacgatttatactttatgcgaagcaaaattattcgttgaattattaacagaattgcgttcttgctctgctgcatctgatttcgatgaggttgttaaaggatatggaaaggatgatacaaggtctgagaacggcaggataaatgctattttagcaaaagcatttaacccttgggttaaatcatttttcggcgatgaccgtcgtgtttataaagatagccgcgctatttacgctcgcatcgcttatgagatgttcttccgcgtcgatccacggtggaaaaacgtcgacgaggatgtgttcttcatggagattctcggacacgacgatgagaacacccagctgcactataagcagttcaagctggccaacttctccagaacctggcgacctgaagttggggatgaaaacaccaggctggtggctctgcagaaactggacgatgaaatgccaggctttgccagaggtgacgctggcgtccgtctccatgaaaccgttaagcagctggtggagcaggacccatcagcaaaaataaccaacagcactctccgggcctttaaatttagcccgacgatgattagccggtacctggagtttgccgctgatgcattggggcagttcgttggcgagaacgggcagtggcagctgaagatagagacacctgcaatcgtcctgcctgatgaagaatccgttgagaccatcgacgaaccggatgatgagtcccaagacgacgagctggatgaagatgaaattgagctcgacgagggtggcggcgatgaaccaaccgaagaggaagggccagaagaacatcagccaactgctctaaaacccgtcttcaagcctgcaaaaaataacggggacggaacgtacaagatagagtttgaatacgatggaaagcattatgcctggtccggccccgccgatagccctatggccgcaatgcgatccgcatgggaaacgtactacagcggtggtggtagcggtggtggtagcggtggtggtagcatgaaaaacatcaaaaaaaaccaggtaatgaacctgggtccgaactctaaactgctgaaagaatacaaatcccagctgatcgaactgaacatcgaacagttcgaagcaggtatcggtctgatcctgggtgatgcttacatccgttctcgtgatgaaggtaaaacctactgtatgcagttcgagtggaaaaacaaagcatacatggaccacgtatgtctgctgtacgatcagtgggtactgtccccgccgcacaaaaaagaacgtgttaaccacctgggtaacctggtaatcacctggggcgcccagactttcaaacaccaagctttcaacaaactggctaacctgttcatcgttaacaacaaaaaaaccatcccgaacaacctggttgaaaactacctgaccccgatgtctctggcatactggttcatggatgatggtggtaaatgggattacaacaaaaactctaccaacaaatcgatcgtactgaacacccagtctttcactttcgaagaagtagaatacctggttaagggtctgcgtaacaaattccaactgaactgttacgtaaaaatcaacaaaaacaaaccgatcatctacatcgattctatgtcttacctgatcttctacaacctgatcaaaccgtacctgatcccgcagatgatgtacaaactgccgaacactatctcctccgaaactttcctgaaataa

SEQ ID NO: 2 - DNA, 1896 bp, Escherichia coli phage N15
  source 1..1896: mol_type = other DNA
atgagcaaggtaaaaatcggtgagttgatcaacacgcttgtgaatgaggtagaggcaattgatgcctcagaccgcccacaaggcgacaaaacgaagagaattaaagccgcagccgcacggtataagaacgcgttatttaatgataaaagaaagttccgtgggaaaggattgcagaaaagaataaccgcgaatacttttaacgcctatatgagcagggcaagaaagcggtttgatgataaattacatcatagctttgataaaaatattaataaattatcggaaaagtatcctctttacagcgaagaattatcttcatggctttctatgcctacggctaatattcgccagcacatgtcatcgttacaatctaaattgaaagaaataatgccgcttgccgaagagttatcaaatgtaagaataggctctaaaggcagtgatgcaaaaatagcaagactaataaaaaaatatccagattggagttttgctcttagtgatttaaacagtgatgattggaaggagcgccgtgactatctttataagttattccaacaaggctctgcgttgttagaagaactacaccagctcaaggtcaaccatgaggttctgtaccatctgcagctaagccctgcggagcgtacatctatacagcaacgatgggccgatgttctgcgcgagaagaagcgtaatgttgtggttattgactacccaacatacatgcagtctatctatgatattttgaataatcctgcgactttatttagtttaaacactcgttctggaatggcacctttggcctttgctctggctgcggtatcagggcgaagaatgattgagataatgtttcagggtgaatttgccgtttcaggaaagtatacggttaatttctcagggcaagctaaaaaacgctctgaagataaaagcgtaaccagaacgatttatactttatgcgaagcaaaattattcgttgaattattaacagaattgcgttcttgctctgctgcatctgatttcgatgaggttgttaaaggatatggaaaggatgatacaaggtctgagaacggcaggataaatgctattttagcaaaagcatttaacccttgggttaaatcatttttcggcgatgaccgtcgtgtttataaagatagccgcgctatttacgctcgcatcgcttatgagatgttcttccgcgtcgatccacggtggaaaaacgtcgacgaggatgtgttcttcatggagattctcggacacgacgatgagaacacccagctgcactataagcagttcaagctggccaacttctccagaacctggcgacctgaagttggggatgaaaacaccaggctggtggctctgcagaaactggacgatgaaatgccaggctttgccagaggtgacgctggcgtccgtctccatgaaaccgttaagcagctggtggagcaggacccatcagcaaaaataaccaacagcactctccgggcctttaaatttagcccgacgatgattagccggtacctggagtttgccgctgatgcattggggcagttcgttggcgagaacgggcagtggcagctgaagatagagacacctgcaatcgtcctgcctgatgaagaatccgttgagaccatcgacgaaccggatgatgagtcccaagacgacgagctggatgaagatgaaattgagctcgacgagggtggcggcgatgaaccaaccgaagaggaagggccagaagaacatcagccaactgctctaaaacccgtcttcaagcctgcaaaaaataacggggacggaacgtacaagatagagtttgaatacgatggaaagcattatgcctggtccggccccgccgatagccctatggccgcaatgcgatccgcatgggaaacgtactacagctaa

SEQ ID NO: 3 - DNA, 56 bp, synthetic construct
  source 1..56: mol_type = other DNA
tatcagcacacaattgcccattatacgcgcgtataatggactattgtgtgctgata

SEQ ID NO: 4 - DNA, 708 bp, Saccharomyces cerevisiae
  source 1..708: mol_type = other DNA
atgaaaaacatcaaaaaaaaccaggtaatgaacctgggtccgaactctaaactgctgaaagaatacaaatcccagctgatcgaactgaacatcgaacagttcgaagcaggtatcggtctgatcctgggtgatgcttacatccgttctcgtgatgaaggtaaaacctactgtatgcagttcgagtggaaaaacaaagcatacatggaccacgtatgtctgctgtacgatcagtgggtactgtccccgccgcacaaaaaagaacgtgttaaccacctgggtaacctggtaatcacctggggcgcccagactttcaaacaccaagctttcaacaaactggctaacctgttcatcgttaacaacaaaaaaaccatcccgaacaacctggttgaaaactacctgaccccgatgtctctggcatactggttcatggatgatggtggtaaatgggattacaacaaaaactctaccaacaaatcgatcgtactgaacacccagtctttcactttcgaagaagtagaatacctggttaagggtctgcgtaacaaattccaactgaactgttacgtaaaaatcaacaaaaacaaaccgatcatctacatcgattctatgtcttacctgatcttctacaacctgatcaaaccgtacctgatcccgcagatgatgtacaaactgccgaacactatctcctccgaaactttcctgaaataa

SEQ ID NO: 5 - DNA, 74 bp, synthetic construct
  source 1..74: mol_type = other DNA
tagggataacagggtaattatcagcacacaattgcccattatacgcgcgtataatggactattgtgtgctgata

SEQ ID NO: 6 - DNA, 76 bp, synthetic construct
  source 1..76: mol_type = other DNA
tagggataacagggtaattttatcagcacacaattgcccattatacgcgcgtataatggactattgtgtgctgata

SEQ ID NO: 7 - DNA, 78 bp, synthetic construct
  source 1..78: mol_type = other DNA
tagggataacagggtaattttttatcagcacacaattgcccattatacgcgcgtataatggactattgtgtgctgata

SEQ ID NO: 8 - DNA, 80 bp, synthetic construct
  source 1..80: mol_type = other DNA
tagggataacagggtaattttttttatcagcacacaattgcccattatacgcgcgtataatggactattgtgtgctgata

SEQ ID NO: 9 - DNA, 82 bp, synthetic construct
  source 1..82: mol_type = other DNA
tagggataacagggtaattttttttttatcagcacacaattgcccattatacgcgcgtataatggactattgtgtgctgata

SEQ ID NO: 10 - skipped

SEQ ID NO: 11 - DNA, 1143 bp, synthetic construct
  source 1..1143: mol_type = other DNA
gctaatcttatggataaaaatgctatggcatagcaaagtgtgacgccgtgcaaataatcaatgtggacttttctgccgtgattatagacacttttgttacgcgtttttgtcatggctttggtcccgctttgttacagaatgcttttaataagcggggttaccggtttggttagcgagaagagccagtaaaagacgcagtgacggcaatgtctgatgcaatatggacaattggtttcttctctgaatggcgggagtatgaaaagtatggctgaagcgcaaaatgatcccctgctgccgggatactcgtttaatgcccatctggtggcgggtttaacgccgattgaggccaacggttatctcgatttttttatcgaccgaccgctgggaatgaaaggttatattctcaatctcaccattcgcggtcagggggtggtgaaaaatcagggacgagaatttgtttgccgaccgggtgatattttgctgttcccgccaggagagattcatcactacggtcgtcatccggaggctcgcgaatggtatcaccagtgggtttactttcgtccgcgcgcctactggcatgaatggcttaactggccgtcaatatttgccaatacggggttctttcgcccggatgaagcgcaccagccgcatttcagcgacctgtttgggcaaatcattaacgccgggcaaggggaagggcgctattcggagctgctggcgataaatctgcttgagcaattgttactgcggcgcatggaagcgattaacgagtcgctccatccaccgatggataatcgggtacgcgaggcttgtcagtacatcagcgatcacctggcagacagcaattttgatatcgccagcgtcgcacagcatgtttgcttgtcgccgtcgcgtctgtcacatcttttccgccagcagttagggattagcgtcttaagctggcgcgaggaccaacgtatcagccaggcgaagctgcttttgagcaccacccggatgcctatcgccaccgtcggtcgcaatgttggttttgacgatcaactctatttctcgcgggtatttaaaaaatgcaccggggccagcccgagcgagttccgtgccggttgtgaagaaaaagtgaatgatgtagccgtcaagttgtcataa

SEQ ID NO: 12 - DNA, 55 bp, synthetic construct
  source 1..55: mol_type = other DNA
tacctgacgctttttatcgcaactctctactgtttctccatacccgtttttttgg

SEQ ID NO: 13 - DNA, 299 bp, synthetic construct
  source 1..299: mol_type = other DNA
aagaaaccaattgtccatattgcatcagacattgccgtcactgcgtcttttactggctcttctcgctaaccaaaccggtaaccccgcttattaaaagcattctgtaacaaagcgggaccaaagccatgacaaaaacgcgtaacaaaagtgtctataatcacggcagaaaagtccacattgattatttgcacggcgtcacactttgctatgccatagcatttttatccataagattagcggatcctacctgacgctttttatcgcaactctctactgtttctccatacccgtttttttgg

SEQ ID NO: 14 - DNA, 24 bp, synthetic construct
  source 1..24: mol_type = other DNA
atgagcaaggtaaaaatcggtgag

SEQ ID NO: 15 - DNA, 23 bp, synthetic construct
  source 1..23: mol_type = other DNA
ttagctgtagtacgtttcccatg

SEQ ID NO: 16 - DNA, 30 bp, synthetic construct
  source 1..30: mol_type = other DNA
atgaaaaacatcaaaaaaaaccaggtaatg

SEQ ID NO: 17 - DNA, 23 bp, synthetic construct
  source 1..23: mol_type = other DNA
ttatttcaggaaagtttcggagg

SEQ ID NO: 18 - DNA, 27 bp, synthetic construct
  source 1..27: mol_type = other DNA
gctaatcttatggataaaaatgctatg

SEQ ID NO: 19 - DNA, 24 bp, synthetic construct
  source 1..24: mol_type = other DNA
ttatgacaacttgacggctacatc

SEQ ID NO: 20 - DNA, 26 bp, synthetic construct
  source 1..26: mol_type = other DNA
aagaaaccaattgtccatattgcatc

SEQ ID NO: 21 - DNA, 25 bp, synthetic construct
  source 1..25: mol_type = other DNA
ccaaaaaaacgggtatggagaaaca

SEQ ID NO: 22 - DNA, 1866 bp, synthetic construct
  source 1..1866: mol_type = other DNA
atgccggggttttacgagattgtgattaaggtccccagcgaccttgacgagcatctgcccggcatttctgacagctttgtgaactgggtggccgagaaggaatgggagttgccgccagattctgacatggatctgaatctgattgagcaggcacccctgaccgtggccgagaagctgcagcgcgactttctgacggaatggcgccgtgtgagtaaggccccggaggcccttttctttgtgcaatttgagaagggagagagctacttccacatgcacgtgctcgtggaaaccaccggggtgaaatccatggttttgggacgtttcctgagtcagattcgcgaaaaactgattcagagaatttaccgcgggatcgagccgactttgccaaactggttcgcggtcacaaagaccagaaatggcgccggaggcgggaacaaggtggtggatgagtgctacatccccaattacttgctccccaaaacccagcctgagctccagtgggcgtggactaatatggaacagtatttaagcgcctgtttgaatctcacggagcgtaaacggttggtggcgcagcatctgacgcacgtgtcgcagacgcaggagcagaacaaagagaatcagaatcccaattctgatgcgccggtgatcagatcaaaaacttcagccaggtacatggagctggtcgggtggctcgtggacaaggggattacctcggagaagcagtggatccaggaggaccaggcctcatacatctccttcaatgcggcctccaactcgcggtcccaaatcaaggctgccttggacaatgcgggaaagattatgagcctgactaaaaccgcccccgactacctggtgggccagcagcccgtggaggacatttccagcaatcggatttataaaattttggaactaaacgggtacgatccccaatatgcggcttccgtctttctgggatgggccacgaaaaagttcggcaagaggaacaccatctggctgtttgggcctgcaactaccgggaagaccaacatcgcggaggccatagcccacactgtgcccttctacgggtgcgtaaactggaccaatgagaactttcccttcaacgactgtgtcgacaagatggtgatctggtgggaggaggggaagatgaccgccaaggtcgtggagtcggccaaagccattctcggaggaagcaaggtgcgcgtggaccagaaatgcaagtcctcggcccagatagacccgactcccgtgatcgtcacctccaacaccaacatgtgcgccgtgattgacgggaactcaacgaccttcgaacaccagcagccgttgcaagaccggatgttcaaatttgaactcacccgccgtctggatcatgactttgggaaggtcaccaagcaggaagtcaaagactttttccggtgggcaaaggatcacgtggttgaggtggagcatgaattctacgtcaaaaagggtggagccaagaaaagacccgcccccagtgacgcagatataagtgagcccaaacgggtgcgcgagtcagttgcgcagccatcgacgtcagacgcggaagcttcgatcaactacgcagacaggtaccaaaacaaatgttctcgtcacgtgggcatgaatctgatgctgtttccctgcagacaatgcgagagaatgaatcagaattcaaatatctgcttcactcacggacagaaagactgtttagagtgctttcccgtgtcagaatctcaacccgtttctgtcgtcaaaaaggcgtatcagaaactgtgctacattcatcatatcatgggaaaggtgccagacgcttgcactgcctgcgatctggtcaatgtggatttggatgactgcatctttgaacaataa

SEQ ID NO: 23 - DNA, 2208 bp, synthetic construct
  source 1..2208: mol_type = other DNA
atggctgccgatggttatcttccagattggctcgaggacactctctctgaaggaataagacagtggtggaagctcaaacctggcccaccaccaccaaagcccgcagagcggcataaggacgacagcaggggtcttgtgcttcctgggtacaagtacctcggacccttcaacggactcgacaagggagagccggtcaacgaggcagacgccgcggccctcgagcacgacaaagcctacgaccggcagctcgacagcggagacaacccgtacctcaagtacaaccacgccgacgcggagtttcaggagcgccttaaagaagatacgtcttttgggggcaacctcggacgagcagtcttccaggcgaaaaagagggttcttgaacctctgggcctggttgaggaacctgttaagacggctccgggaaaaaagaggccggtagagcactctcctgtggagccagactcctcctcgggaaccggaaaggcgggccagcagcctgcaagaaaaagattgaattttggtcagactggagacgcagactcagtacctgacccccagcctctcggacagccaccagcagccccctctggtctgggaactaatacgatggctacaggcagtggcgcaccaatggcagacaataacgagggcgccgacggagtgggtaattcctcgggaaattggcattgcgattccacatggatgggcgacagagtcatcaccaccagcacccgaacctgggccctgcccacctacaacaaccacctctacaaacaaatttccagccaatcaggagcctcgaacgacaatcactactttggctacagcaccccttgggggtattttgacttcaacagattccactgccacttttcaccacgtgactggcaaagactcatcaacaacaactggggattccgacccaagagactcaacttcaagctctttaacattcaagtcaaagaggtcacgcagaatgacggtacgacgacgattgccaataaccttaccagcacggttcaggtgtttactgactcggagtaccagctcccgtacgtcctcggctcggcgcatcaaggatgcctcccgccgttcccagcagacgtcttcatggtgccacagtatggatacctcaccctgaacaacgggagtcaggcagtaggacgctcttcattttactgcctggagtactttccttctcagatgctgcgtaccggaaacaactttaccttcagctacacttttgaggacgttcctttccacagcagctacgctcacagccagagtctggaccgtctcatgaatcctctcatcgaccagtacctgtattacttgagcagaacaaacactccaagtggaaccaccacgcagtcaaggcttcagttttctcaggccggagcgagtgacattcgggaccagtctaggaactggcttcctggaccctgttaccgccagcagcgagtatcaaagacatctgcggataacaacaacagtgaatactcgtggactggagctaccaagtaccacctcaatggcagagactctctggtgaatccgggcccggccatggcaagccacaaggacgatgaagaaaagttttttcctcagagcggggttctcatctttgggaagcaaggctcagagaaaacaaatgtggacattgaaaaggtcatgattacagacgaagaggaaatcaggacaaccaatcccgtggctacggagcagtatggttctgtatctaccaacctccagagaggcaacagacaagcagctaccgcagatgtcaacacacaaggcgttcttccaggcatggtctggcaggacagagatgtgtaccttcaggggcccatctgggcaaagattccacacacggacggacattttcacccctctcccctcatgggtggattcggacttaaacaccctcctccacagattctcatcaagaacaccccggtacctgcgaatccttcgaccaccttcagtgcggcaaagtttgcttccttcatcacacagtactccacgggacaggtcagcgtggagatcgagtgggagctgcagaaggaaaacagcaaacgctggaatcccgaaattcagtacacttccaactacaacaagtctgttaatgtggactttactgtggacactaatggcgtgtattcagagcctcgccccattggcaccagatacctgactcgtaatctgtaa

SEQ ID NO: 24 - protein, 631 aa, Escherichia coli phage N15
MSKVKIGELINTLVNEVEAIDASDRPQGDKTKRIKAAAARYKNALFNDKRKFRGKGLQKRITANTFNAYMSRARKRFDDKLHHSFDKNINKLSEKYPLYSEELSSWLSMPTANIRQHMSSLQSKLKEIMPLAEELSNVRIGSKGSDAKIARLIKKYPDWSFALSDLNSDDWKERRDYLYKLFQQGSALLEELHQLKVNHEVLYHLQLSPAERTSIQQRWADVLREKKRNVVVIDYPTYMQSIYDILNNPATLFSLNTRSGMAPLAFALAAVSGRRMIEIMFQGEFAVSGKYTVNFSGQAKKRSEDKSVTRTIYTLCEAKLFVELLTELRSCSAASDFDEVVKGYGKDDTRSENGRINAILAKAFNPWVKSFFGDDRRVYKDSRAIYARIAYEMFFRVDPRWKNVDEDVFFMEILGHDDENTQLHYKQFKLANFSRTWRPEVGDENTRLVALQKLDDEMPGFARGDAGVRLHETVKQLVEQDPSAKITNSTLRAFKFSPTMISRYLEFAADALGQFVGENGQWQLKIETPAIVLPDEESVETIDEPDDESQDDELDEDEIELDEGGGDEPTEEEGPEEHQPTALKPVFKPAKNNGDGTYKIEFEYDGKHYAWSGPADSPMAAMRSAWETYYS

SEQ ID NO: 25 - protein, 235 aa, Saccharomyces cerevisiae
MKNIKKNQVMNLGPNSKLLKEYKSQLIELNIEQFEAGIGLILGDAYIRSRDEGKTYCMQFEWKNKAYMDHVCLLYDQWVLSPPHKKERVNHLGNLVITWGAQTFKHQAFNKLANLFIVNNKKTIPNNLVENYLTPMSLAYWFMDDGGKWDYNKNSTNKSIVLNTQSFTFEEVEYLVKGLRNKFQLNCYVKINKNKPIIYIDSMSYLIFYNLIKPYLIPQMMYKLPNTISSETFLK

SEQ ID NO: 26 - DNA, 32 bp, synthetic construct
  source 1..32: mol_type = other DNA
cataataacaatatcatgatattgttattatg

SEQ ID NO: 27 - DNA, 90 bp, synthetic construct
  source 1..90: mol_type = other DNA
cctatattgggccacctatgtatgcacagttcgcccatactatacgtatagtatgggcgaactgtgcatacataggtggcccaatatagg

SEQ ID NO: 28 - DNA, 90 bp, synthetic construct
  source 1..90: mol_type = other DNA
gggatcccgttccatacatacatgtatccatgtggcatactatacgtatagtatgccgatgttacatatggtatcattcgggatcccgtt

SEQ ID NO: 29 - DNA, 44 bp, synthetic construct
  source 1..44: mol_type = other DNA
cacacaattgcccattatacgcgcgtataatgggcaattgtgtg

SEQ ID NO: 30 - DNA, 42 bp, synthetic construct
  source 1..42: mol_type = other DNA
acctatttcagcatactacgcgcgtagtatgctgaaataggt

SEQ ID NO: 31 - DNA, 18 bp, synthetic construct
  source 1..18: mol_type = other DNA
attaccctgttatcccta

SEQ ID NO: 32 - DNA, 27 bp, synthetic construct
  source 1..27: mol_type = other DNA
taactataacggtcctaaggtagcgaa

SEQ ID NO: 33 - DNA, 22 bp, synthetic construct
  source 1..22: mol_type = other DNA
caaaacgtcgtgagacagtttc

SEQ ID NO: 34 - DNA, 36 bp, synthetic construct
  source 1..36: mol_type = other DNA
ggtggtggtagcggtggtggtagcggtggtggtagc

SEQ ID NO: 35 - DNA, 816 bp, unidentified
  source 1..816: mol_type = unassigned DNA
atgagccatattcaacgggaaacgtcttgctctaggccgcgattaaattccaacatggatgctgatttatatgggtataaatgggctcgcgataatgtcgggcaatcaggtgcgacaatctatcgattgtatgggaagcccgatgcgccagagttgtttctgaaacatggcaaaggtagcgttgccaatgatgttacagatgagatggtcagactaaactggctgacggaatttatgcctcttccgaccatcaagcattttatccgtactcctgatgatgcatggttactcaccactgcgatccccgggaaaacagcattccaggtattagaagaatatcctgattcaggtgaaaatattgttgatgcgctggcagtgttcctgcgccggttgcattcgattcctgtttgtaattgtccttttaacagcgatcgcgtatttcgtctcgctcaggcgcaatcacgaatgaataacggtttggttgatgcgagtgattttgatgacgagcgtaatggctggcctgttgaacaagtctggaaagaaatgcataaacttttgccattctcaccggattcagtcgtcactcatggtgatttctcacttgataaccttatttttgacgaggggaaattaataggttgtattgatgttggacgagtcggaatcgcagaccgataccaggatcttgccatcctatggaactgcctcggtgagttttctccttcattacagaaacggctttttcaaaaatatggtattgataatcctgatatgaataaattgcagtttcatttgatgctcgatgagtttttctaa

SEQ ID NO: 36 - DNA, 20 bp, synthetic construct
  source 1..20: mol_type = other DNA
taacccgggcgtttaaacag

SEQ ID NO: 37 - DNA, 35 bp, synthetic construct
  source 1..35: mol_type = other DNA
gtttaaacgcccgggttagctgtagtacgtttccc

SEQ ID NO: 38 - DNA, 35 bp, synthetic construct
  source 1..35: mol_type = other DNA
gacaattggtttcttattaccctgttatccctaat